European Patent Specification EP 3 908 677 B1, published May 1, 2024. Title: METHOD. Applicant: 3CR Bioscience Ltd. The sequence listing filed with the application follows.

SEQUENCE LISTING (20 sequences)

SEQ ID NO: 1 - DNA, 50 bp, Artificial Sequence
  Synthetic oligonucleotide
gaaggtgaccaagttcatgctgaagctccacaatttggtgaattatcaat

SEQ ID NO: 2 - DNA, 50 bp, Artificial Sequence
  Synthetic oligonucleotide
gaaggtcggagtcaacggattgaagctccacaatttggtgaattatcaaa

SEQ ID NO: 3 - DNA, 29 bp, Artificial Sequence
  Synthetic oligonucleotide
cactctagtactatatctgtcacatggta

SEQ ID NO: 4 - DNA, 21 bp, Artificial Sequence
  Synthetic oligonucleotide
  misc_feature: 5' 56-FAM
  misc_feature: 3' 3IABkFQ
gaaggtgaccaagttcatgct

SEQ ID NO: 5 - DNA, 21 bp, Artificial Sequence
  Synthetic oligonucleotide
  misc_feature: 5' 5HEX
  misc_feature: 3' 3IABkFQ
gaaggtcggagtcaacggatt

SEQ ID NO: 6 - DNA, 21 bp, Artificial Sequence
  Synthetic oligonucleotide
gaaggtgaccaagttcatgct

SEQ ID NO: 7 - DNA, 21 bp, Artificial Sequence
  Synthetic oligonucleotide
gaaggtcggagtcaacggatt

SEQ ID NO: 8 - DNA, 42 bp, Artificial Sequence
  Synthetic oligonucleotide
gaaggtgaccaagttcatgctgaaggtgaccaagttcatgct

SEQ ID NO: 9 - DNA, 42 bp, Artificial Sequence
  Synthetic oligonucleotide
gaaggtcggagtcaacggattgaaggtcggagtcaacggatt

SEQ ID NO: 10 - DNA, 41 bp, Artificial Sequence
  Synthetic oligonucleotide
gaaggtgaccaagttcatgctgagtgcaggttcagacgtcc

SEQ ID NO: 11 - DNA, 22 bp, Artificial Sequence
  Synthetic oligonucleotide
ctcccttccacctccgtaccat

SEQ ID NO: 12 - DNA, 43 bp, Artificial Sequence
  Synthetic oligonucleotide
gaaggtcggagtcaacggattctgagtgcaggttcagacgtct

SEQ ID NO: 13 - DNA, 401 bp, Homo sapiens
tgtctagctagctagccttccatcagccatcttcttttttcattgtcagtgcctctttatgaaggtaaaattgacataccagaacatatcctcattttaggcacacatttcatgatttaagtaaatttatacagttgtgcaaccatcagcataatctagttttagaacacttctgttaccctaagcacgttctcctcataycgtttgtcgtcaatccctaccacggctaccagtctcaggcagctactaatctatctgctttttttctgtgtaattttgccttttccagaaagtctttatagatagaagtatacaatgtatagtctcttctgtttggcttctttcattagaatggtgcttttgagattcatctatgttgtggcatgtatcagtaggttgtt

SEQ ID NO: 14 - DNA, 51 bp, Artificial Sequence
  Synthetic oligonucleotide
agctgctattgttaccagtgacgcagctccctaagcacgttctcctcatac

SEQ ID NO: 15 - DNA, 52 bp, Artificial Sequence
  Synthetic oligonucleotide
tggccagtgtattctgcacaggtggccaaccctaagcacgttctcctcatat

SEQ ID NO: 16 - DNA, 22 bp, Artificial Sequence
  Synthetic oligonucleotide
gactggtagccgtggtagggat

SEQ ID NO: 17 - DNA, 28 bp, Artificial Sequence
  Synthetic oligonucleotide
  misc_feature: 5' 6-FAM
  misc_feature: 3' IABkFQ
agctgctattgttaccagtgacgcagct

SEQ ID NO: 18 - DNA, 28 bp, Artificial Sequence
  Synthetic oligonucleotide
  misc_feature: 5' HEX
  misc_feature: 3' IABkFQ
tggccagtgtattctgcacaggtggcca

SEQ ID NO: 19 - DNA, 27 bp, Artificial Sequence
  Synthetic oligonucleotide
gctgctattgttaccagtgacgcagct

SEQ ID NO: 20 - DNA, 27 bp, Artificial Sequence
  Synthetic oligonucleotide
ggccagtgtattctgcacaggtggcca